European Patent Specification EP 3 895 717 B1, published August 7, 2024. Title: Pharmaceutical composition for prevention or treatment of cancer comprising Weissella cibaria WIKIM28 as active ingredient. Applicant: Korea Food Research Institute. The sequence listing filed with the application follows.

SEQUENCE LISTING (1 sequence)

SEQ ID NO: 1 - DNA, 1508 bp, Weissella cibaria WIKIM28
ggatgacgctggcggcgtgcctaatacatgcaagtcgaacgctttgtggttcaactgatttgaagagcttgctcagatatgacgatggacattgcaaagagtggcgaacgggtgagtaacacgtgggaaacctacctcttagcaggggataacatttggaaacagatgctaataccgtataacaatagcaaccgcatggttgctacttaaaagatggttctgctatcactaagagatggtcccgcggtgcattagttagttggtgaggtaatggctcaccaagacgatgatgcatagccgagttgagagactgatcggccacaatgggactgagacacggcccatactcctacgggaggcagcagtagggaatcttccacaatgggcgaaagcctgatggagcaacgccgcgtgtgtgatgaagggtttcggctcgtaaaacactgttgtaagagaagaatgacattgagagtaactgttcaatgtgtgacggtatcttaccagaaaggaacggctaaatacgtgccagcagccgcggtaatacgtatgttccaagcgttatccggatttattgggcgtaaagcgagcgcagacggttatttaagtctgaagtgaaagccctcagctcaactgaggaattgctttggaaactggatgacttgagtgcagtagaggaaagtggaactccatgtgtagcggtgaaatgcgtagatatatggaagaacaccagtggcgaaggcggctttctggactgtaactgacgttgaggctcgaaagtgtgggtagcaaacaggattagataccctggtagtccacaccgtaaacgatgagtgctaggtgtttgagggtttccgcccttaagtgccgcagctaacgcattaagcactccgcctggggagtacgaccgcaaggttgaaactcaaaggaattgacggggacccgcacaagcggtggagcatgtggtttaattcgaagcaacgcgaagaaccttaccaggtcttgacatcccttgacaactccagagatggagcgttcccttcggggacaaggtgacaggtggtgcatggttgtcgtcagctcgtgtcgtgagatgttgggttaagtcccgcaacgagcgcaacccttattactagttgccagcatttagttgggcactctagtgagactgccggtgacaaaccggaggaaggtggggatgacgtcaaatcatcatgccccttatgacctgggctacacacgtgctacaatggcgtatacaacgagttgccaacccgcgagggtgagctaatctcttaaagtacgtctcagttcggattgtaggctgcaactcgcctacatgaagtcggaatcgctagtaatcgcggatcagcacgccgcggtgaatacgttcccgggtcttgtacacaccgcccgtcacaccatgagagtttgtaacacccaaagccggtggggtaaccttcgggagccagccgtctaaggtgggacagatgattagggtgaagtctaca